European Patent Specification EP 3 760 713 B1, published July 8, 2026. Title: LIPASE VARIANTS AND POLYNUCLEOTIDES ENCODING SAME. Applicant: Novozymes A/S. The sequence listing filed with the application follows.

SEQUENCE LISTING (3 sequences)

SEQ ID NO: 1 - DNA, 1098 bp, Rhizomucor miehei
  CDS (1)..(1098)
  sig_peptide (1)..(72)
  mat_peptide (292)..(1098)
atggttctcaagcagcgtgcaaactacctaggatttctgattgtattcttcacggccttcctggtggaagcggtacccatcaagagacaatcgaattccacggtcgacagtctgccgcctgcctcggtcctcatcccctcgagaacctcggcaccttcatcatcaccaagcacaaccgaccctgaagctccagccatgagtcgcaatggaccgctgccctcggatgtagagactaaatatggcatggctttgaatgctacttcctatccggattctgtggtccaagcaatgagcattgatggtggtatccgcgctgcgacctcgcaagaaatcaatgaattgacttattacactacactatctgccaactcgtactgccgcactgtcattcctggagctacctgggactgtatccactgtgatgcaacggaggatctcaagattatcaagacttggagcacgctcatctatgatacaaatgcaatggttgcacgtggtgacagcgaaaaaactatctatatcgttttccgaggttcgagctctatccgcaactggattgctgatctcacctttgtgccagtttcatatcctccggtcagtggtacaaaagtacacaagggattcctggacagttacggggaagttcaaaacgagcttgttgctactgttcttgatcaattcaagcaatatccaagctacaaggttgctgttacaggtcactcactcggtggtgctactgcgttgctttgcgccctggatctctatcaacgagaagaaggactctcatccagcaacttgttcctttacactcaaggtcaaccacgggtaggcgaccctgcctttgccaactacgttgttagcaccggcattccttacaggcgcacggtcaatgaacgagatatcgttcctcatcttccacctgctgcttttggttttctccacgctggcgaggagtattggattactgacaatagcccagagactgttcaggtctgcacaagcgatctggaaacctctgattgctctaacagcattgttcccttcacaagtgttcttgaccatctctcgtactttggtatcaacacaggcctctgtact

SEQ ID NO: 2 - protein, 366 aa, Rhizomucor miehei
MVLKQRANYLGFLIVFFTAFLVEAVPIKRQSNSTVDSLPPASVLIPSRTSAPSSSPSTTDPEAPAMSRNGPLPSDVETKYGMALNATSYPDSVVQAMSIDGGIRAATSQEINELTYYTTLSANSYCRTVIPGATWDCIHCDATEDLKIIKTWSTLIYDTNAMVARGDSEKTIYIVFRGSSSIRNWIADLTFVPVSYPPVSGTKVHKGFLDSYGEVQNELVATVLDQFKQYPSYKVAVTGHSLGGATALLCALDLYQREEGLSSSNLFLYTQGQPRVGDPAFANYVVSTGIPYRRTVNERDIVPHLPPAAFGFLHAGEEYWITDNSPETVQVCTSDLETSDCSNSIVPFTSVLDHLSYFGINTGLCT

SEQ ID NO: 3 - protein, 269 aa, Rhizomucor miehei
SIDGGIRAATSQEINELTYYTTLSANSYCRTVIPGATWDCIHCDATEDLKIIKTWSTLIYDTNAMVARGDSEKTIYIVFRGSSSIRNWIADLTFVPVSYPPVSGTKVHKGFLDSYGEVQNELVATVLDQFKQYPSYKVAVTGHSLGGATALLCALDLYQREEGLSSSNLFLYTQGQPRVGDPAFANYVVSTGIPYRRTVNERDIVPHLPPAAFGFLHAGEEYWITDNSPETVQVCTSDLETSDCSNSIVPFTSVLDHLSYFGINTGLCT